European Patent Specification EP 4 017 998 B1, published November 6, 2024. Title: MULTI-SITE ENRICHMENT OF DELETIONS IN DNA MICROSATELLITES. Applicant: Dana-Farber Cancer Institute, Inc. Application Not Yet Assigned. The sequence listing filed with the application follows.

SEQUENCE LISTING (8 sequences)

SEQ ID NO: 1 - DNA, 20 bp, Unknown
  may be derived from multiple organisms
  modified_base (2)..(2): may be modified by an LNA-containing deoxy-thymidine or any other modified version of deoxy-thymidine
  modified_base (19)..(19): may be modified by an LNA-containing deoxy-thymidine or any other modified version of deoxy-thymidine
tttttttttttttttttttt

SEQ ID NO: 2 - DNA, 19 bp, Unknown
  may be derived from any organism
aaaaaaaaaaaaaaaaaaa

SEQ ID NO: 3 - DNA, 31 bp, Artificial Sequence
  Synthetic Polynucloetide
  misc_feature (1)..(7): are inosine
  modified_base (9)..(9): may be modified by an LNA-containing deoxy-thymidine or any other modified version of deoxy-thymidine
  modified_base (26)..(26): may be modified by an LNA-containing deoxy-thymidine or any other modified version of deoxy-thymidine
  misc_feature (28)..(31): are inosine
nnnnnnnttttttttttttttttttttnnnn

SEQ ID NO: 4 - DNA, 22 bp, Artificial Sequence
  Synthetic Polynucleotide
  misc_feature (1)..(5): are inosine
  misc_feature (21)..(22): are insosine
nnnnnaaaaaaaaaaaaaaann

SEQ ID NO: 5 - DNA, 22 bp, Artificial Sequence
  Synthetic Polynucleotide
  misc_feature (1)..(2): are inosine
  modified_base (3)..(3): may be modified by an LNA-containing deoxy-thymidine or any other modified version of deoxy-thymidine
  modified_base (17)..(17): may be modified by an LNA-containing deoxy-thymidine or any other modified version of deoxy-thymidine
  misc_feature (18)..(22): is inosine
nntttttttttttttttnnnnn

SEQ ID NO: 6 - DNA, 480 bp, Homo sapiens
taattgctaagaaaaatcctctcttcctcacaggctcatacatgaaagaggatgtgactcccgccatcatggaggatgacgagttggccctagacttagaagacttgctgagcttttcttaccaggtggcaaagggcatggctttcctcgcctccaagaatgtaagtgggagtgattctctaaagagttttgtgttttgtttttttgatttttttttttttttttttttttttgagaacagagcattttagagccatagttaaaatgcagaatgtcattttgaagtgcggtaaccaaaagcagaggaaatttagtttcttcatgttccaactgctgtctctttggaattcctgttctaatttataagctgtaaagtacaagcctgtctaaatgagtttttctatgaatattcttttatatgcagtgaaattcttttaaaacttttggcttttaggatataggatatgttcctagagaaca

SEQ ID NO: 7 - DNA, 15 bp, Unknown
  may be derived from any organism
acacacacacacaca

SEQ ID NO: 8 - DNA, 18 bp, Unknown
  may be derived from any organism
cagcagcagcagcagcag